European Patent Application EP 4 685 159 A1, published January 28, 2026. Title: Single domain antibodies to CD34 suitable for targeting hematopoietic stem cells. Applicant: PROVIREX Genome Editing Therapies GmbH. Application EP. The sequence listing filed with the application follows.

SEQUENCE LISTING (80 sequences)

SEQ ID NO: 1 - protein, 5 aa, Vicugna pacos
TFGMN

SEQ ID NO: 2 - protein, 17 aa, Vicugna pacos
  VARIANT 5: note = X may be any naturally occurring amino acid
  VARIANT 9: note = X may be any naturally occurring amino acid
  VARIANT 12: note = X may be any naturally occurring amino acid
  VARIANT 17: note = X may be any naturally occurring amino acid
  VARIANT 10: note = X may be any naturally occurring amino acid
  VARIANT 13: note = X may be any naturally occurring amino acid
  VARIANT 16: note = X may be any naturally occurring amino acid
TISAXGLRXXYXXSVXX

SEQ ID NO: 3 - protein, 17 aa, Vicugna pacos
  VARIANT 5: note = X is a polar amino acid
  VARIANT 9: note = X is a polar or unpolar amino acid
  VARIANT 10: note = X is a basic or polar amino acid
  VARIANT 12: note = X is a polar or unpolar amino acid
  VARIANT 13: note = X is a an acidic amino acid
  VARIANT 17: note = X is an acidic or an unpolar amino acid
TISAXGLRXXYXXSVKX

SEQ ID NO: 4 - protein, 17 aa, Vicugna pacos
  VARIANT 5: note = X is N or T
  VARIANT 9: note = X is T or V
  VARIANT 10: note = X is R or N
  VARIANT 12: note = X is S or A
  VARIANT 13: note = X is D or E
  VARIANT 17: note = X6 is D or G.
TISAXGLRXXYXXSVKX

SEQ ID NO: 5 - protein, 17 aa, Vicugna pacos
TISATGLRVNYAESVKG

SEQ ID NO: 6 - protein, 17 aa, Vicugna pacos
TISANGLRTRYSDSVKD

SEQ ID NO: 7 - protein, 7 aa, Vicugna pacos
GWPSPIY

SEQ ID NO: 8 - protein, 116 aa, Vicugna pacos
EVQLVESGGGLVQPGGSLRLSCAASGLTFSTFGMNWYRQASGKERELVATISATGLRVNYAESVKGRFTVSRDNVKDTVYLQMNSLIPEDTAVYECAAGWPSPIYWGQGTRVTVSS

SEQ ID NO: 9 - protein, 116 aa, Vicugna pacos
HVQLVESGGGLVQPGGSLRLSCAASGLTFSTFGMNWYRQASGKERELVATISANGLRTRYSDSVKDRFTISRDNSKDTVYLQMSSLIPEDTAVYECAAGWPSPIYWGQGAQVTVSS

SEQ ID NO: 10 - protein, 116 aa, Vicugna pacos
HVQLVESGGGLVQPGGSLTLSCVVSGLTFSTYGMTWYREASGKEREFVAYMSNGGLRRNYAESVKDRFTISRDNVKNTVYLQMNSLIPEDTAVYYCAAGWPSPVYWGQGTRVTVSS

SEQ ID NO: 11 - protein, 119 aa, Vicugna pacos
QVQLVESGGGLVQPGGSLRLSCAASGTIFDIYDMDWYRQAPEKQRELVAGVSSDGLTNYADSVKGRFTISRDNAKNTVYLQMNSLKPEDTAVYYCWAGNERAGPSFGSWGQGSPVTVSS

SEQ ID NO: 12 - protein, 124 aa, Vicugna pacos
DVQLVESGGGLVQAGGSLRLSCAASGSIFSIDGMGWYRQAPGKERELVAAISNVGSTYYANSLKGRFAISRDNAKNTVYLQMNSLKPEDTAMYYCAAYRAKTDKESDSETFAAWGQGTQVTVSS

SEQ ID NO: 13 - protein, 118 aa, Vicugna pacos
HVQLVESGGGLVQAGGSLRLSCAASGTIFSISGMGWYREAPGKERELVASISSGGSTYYADSVKGRFTISRDNAKNTLYLQMNSLNAEDTATYYCAALEGRGETFASWGQGAQVTVSS

SEQ ID NO: 14 - protein, 118 aa, Vicugna pacos
DVQLVESGGGLVQAGGSLRLSCAASENIFSIDAMGWYRQAPGKEREVVAVISSGGSTYYGDSVKGRFAISRDNAKNTLFLQMNSLKPEDTAMYYCAALGGIEETFRSWGQGTQVTVSS

SEQ ID NO: 15 - protein, 113 aa, Vicugna pacos
QVQLVESGGGLVQPGGSLRLSCAASGFAFSSYYMHWFRQAPGKEREKVASISNGGGITHYEDSVKGRFTISRDNAKNMVYLEMNSLKPEDTAVYYCKAGTTYWGQGTPVTVSS

SEQ ID NO: 16 - protein, 113 aa, Vicugna pacos
HVQLVESGGGLVQPGGSLRLSCAASGFAFNMYVMRWYRQAPGKERELVATITNGGGITHYEDSVKGRFTISRDNAKNTVYLQMNSLKPEDTAVYYCQAGTTYWGQGTPVTVSS

SEQ ID NO: 17 - protein, 5 aa, Vicugna pacos
TYGMT

SEQ ID NO: 18 - protein, 17 aa, Vicugna pacos
YMSNGGLRRNYAESVKD

SEQ ID NO: 19 - protein, 7 aa, Vicugna pacos
GWPSPVY

SEQ ID NO: 20 - protein, 5 aa, Vicugna pacos
IYDMD

SEQ ID NO: 21 - protein, 16 aa, Vicugna pacos
GVSSDGLTNYADSVKG

SEQ ID NO: 22 - protein, 11 aa, Vicugna pacos
GNERAGPSFGS

SEQ ID NO: 23 - protein, 5 aa, Vicugna pacos
IDGMG

SEQ ID NO: 24 - protein, 16 aa, Vicugna pacos
AISNVGSTYYANSLKG

SEQ ID NO: 25 - protein, 16 aa, Vicugna pacos
YRAKTDKESDSETFAA

SEQ ID NO: 26 - protein, 5 aa, Vicugna pacos
ISGMG

SEQ ID NO: 27 - protein, 16 aa, Vicugna pacos
SISSGGSTYYADSVKG

SEQ ID NO: 28 - protein, 10 aa, Vicugna pacos
LEGRGETFAS

SEQ ID NO: 29 - protein, 5 aa, Vicugna pacos
IDAMG

SEQ ID NO: 30 - protein, 16 aa, Vicugna pacos
VISSGGSTYYGDSVKG

SEQ ID NO: 31 - protein, 10 aa, Vicugna pacos
LGGIEETFRS

SEQ ID NO: 32 - protein, 5 aa, Vicugna pacos
SYYMH

SEQ ID NO: 33 - protein, 17 aa, Vicugna pacos
SISNGGGITHYEDSVKG

SEQ ID NO: 34 - protein, 4 aa, Vicugna pacos
GTTY

SEQ ID NO: 35 - protein, 5 aa, Vicugna pacos
MYVMR

SEQ ID NO: 36 - protein, 17 aa, Vicugna pacos
TITNGGGITHYEDSVKG

SEQ ID NO: 37 - protein, 4 aa, Vicugna pacos
GTTY

SEQ ID NO: 38 - protein, 30 aa, Vicugna pacos
EVQLVESGGGLVQPGGSLRLSCAASGLTFS

SEQ ID NO: 39 - protein, 14 aa, Vicugna pacos
WYRQASGKERELVA

SEQ ID NO: 40 - protein, 32 aa, Vicugna pacos
RFTVSRDNVKDTVYLQMNSLIPEDTAVYECAA

SEQ ID NO: 41 - protein, 11 aa, Vicugna pacos
WGQGTRVTVSS

SEQ ID NO: 42 - protein, 30 aa, Vicugna pacos
HVQLVESGGGLVQPGGSLRLSCAASGLTFS

SEQ ID NO: 43 - protein, 14 aa, Vicugna pacos
WYRQASGKERELVA

SEQ ID NO: 44 - protein, 32 aa, Vicugna pacos
RFTISRDNSKDTVYLQMSSLIPEDTAVYECAA

SEQ ID NO: 45 - protein, 11 aa, Vicugna pacos
WGQGAQVTVSS

SEQ ID NO: 46 - protein, 30 aa, Vicugna pacos
HVQLVESGGGLVQPGGSLTLSCVVSGLTFS

SEQ ID NO: 47 - protein, 14 aa, Vicugna pacos
WYREASGKEREFVA

SEQ ID NO: 48 - protein, 32 aa, Vicugna pacos
RFTISRDNVKNTVYLQMNSLIPEDTAVYYCAA

SEQ ID NO: 49 - protein, 11 aa, Vicugna pacos
WGQGTRVTVSS

SEQ ID NO: 50 - protein, 30 aa, Vicugna pacos
HVQLVESGGGLVQPGGSLRLSCAASGFAFN

SEQ ID NO: 51 - protein, 14 aa, Vicugna pacos
WYRQAPGKERELVA

SEQ ID NO: 52 - protein, 32 aa, Vicugna pacos
RFTISRDNAKNTVYLQMNSLKPEDTAVYYCQA

SEQ ID NO: 53 - protein, 11 aa, Vicugna pacos
WGQGTPVTVSS

SEQ ID NO: 54 - protein, 30 aa, Vicugna pacos
QVQLVESGGGLVQPGGSLRLSCAASGFAFS

SEQ ID NO: 55 - protein, 14 aa, Vicugna pacos
WFRQAPGKEREKVA

SEQ ID NO: 56 - protein, 32 aa, Vicugna pacos
RFTISRDNAKNMVYLEMNSLKPEDTAVYYCKA

SEQ ID NO: 57 - protein, 11 aa, Vicugna pacos
WGQGTPVTVSS

SEQ ID NO: 58 - protein, 30 aa, Vicugna pacos
DVQLVESGGGLVQAGGSLRLSCAASENIFS

SEQ ID NO: 59 - protein, 14 aa, Vicugna pacos
WYRQAPGKEREVVA

SEQ ID NO: 60 - protein, 32 aa, Vicugna pacos
RFAISRDNAKNTLFLQMNSLKPEDTAMYYCAA

SEQ ID NO: 61 - protein, 11 aa, Vicugna pacos
WGQGTQVTVSS

SEQ ID NO: 62 - protein, 30 aa, Vicugna pacos
HVQLVESGGGLVQAGGSLRLSCAASGTIFS

SEQ ID NO: 63 - protein, 14 aa, Vicugna pacos
WYREAPGKERELVA

SEQ ID NO: 64 - protein, 32 aa, Vicugna pacos
RFTISRDNAKNTLYLQMNSLNAEDTATYYCAA

SEQ ID NO: 65 - protein, 11 aa, Vicugna pacos
WGQGAQVTVSS

SEQ ID NO: 66 - protein, 30 aa, Vicugna pacos
DVQLVESGGGLVQAGGSLRLSCAASGSIFS

SEQ ID NO: 67 - protein, 14 aa, Vicugna pacos
WYRQAPGKERELVA

SEQ ID NO: 68 - protein, 32 aa, Vicugna pacos
RFAISRDNAKNTVYLQMNSLKPEDTAMYYCAA

SEQ ID NO: 69 - protein, 11 aa, Vicugna pacos
WGQGTQVTVSS

SEQ ID NO: 70 - protein, 30 aa, Vicugna pacos
QVQLVESGGGLVQPGGSLRLSCAASGTIFD

SEQ ID NO: 71 - protein, 14 aa, Vicugna pacos
WYRQAPEKQRELVA

SEQ ID NO: 72 - protein, 32 aa, Vicugna pacos
RFTISRDNAKNTVYLQMNSLKPEDTAVYYCWA

SEQ ID NO: 73 - protein, 11 aa, Vicugna pacos
WGQGSPVTVSS

SEQ ID NO: 74 - protein, 17 aa, Vicugna pacos
  VARIANT 5: note = X may be any naturally occurring amino acid
  VARIANT 9: note = X may be any naturally occurring amino acid
  VARIANT 10: note = X may be any naturally occurring amino acid
  VARIANT 12: note = X may be any naturally occurring amino acid
  VARIANT 13: note = X may be any naturally occurring amino acid
  VARIANT 17: note = X may be any naturally occurring amino acid
TISAXGLRXXYXXSVKX

SEQ ID NO: 75 - protein, 17 aa, Vicugna pacos
  VARIANT 5: note = X is a polar amino acid
  VARIANT 9: note = X is a polar or unpolar amino acid
  VARIANT 10: note = X is a basic or polar amino acid
  VARIANT 12: note = X is a polar or unpolar amino acid
  VARIANT 16: note = X is K or R
  VARIANT 17: note = X is an acidic or an unpolar amino acid
TISAXGLRXXYXXSVXX

SEQ ID NO: 76 - protein, 17 aa, Vicugna pacos
  VARIANT 5: note = X is N or T
  VARIANT 9: note = X is T or V
  VARIANT 10: note = X is R or N
  VARIANT 12: note = X is S orA
  VARIANT 13: note = X is D or E
  VARIANT 16: note = X is K or R
  VARIANT 17: note = X is D or G
TISAXGLRXXYXXSVXX

SEQ ID NO: 77 - protein, 17 aa, Vicugna pacos
  VARIANT 16: note = X is R or K, optionally R
TISATGLRVNYAESVXG

SEQ ID NO: 78 - protein, 17 aa, Vicugna pacos
  VARIANT 16: note = X is R or K, optionally R
TISANGLRTRYSDSVXD

SEQ ID NO: 79 - protein, 116 aa, Vicugna pacos
EVQLVESGGGLVQPGGSLRLSCAASGLTFSTFGMNWYRQASGRERELVATISATGLRVNYAESVRGRFTVSRDNVRDTVYLQMNSLIPEDTAVYECAAGWPSPIYWGQGTRVTVSS

SEQ ID NO: 80 - protein, 116 aa, Vicugna pacos
HVQLVESGGGLVQPGGSLRLSCAASGLTFSTFGMNWYRQASGRERELVATISANGLRTRYSDSVRDRFTISRDNSRDTVYLQMSSLIPEDTAVYECAAGWPSPIYWGQGAQVTVSS